European Patent Application EP 4 273 173 A1, published November 8, 2023. Title: LONG-ACTING INTERLEUKIN-15 FUSION PROTEIN, PREPARATION METHOD THEREFOR, AND APPLICATION THEREOF. Applicant: Suzhou Forlong Biotechnology Co., Ltd. Application EP 21912542.4. The sequence listing filed with the application follows.

SEQUENCE LISTING (4 sequences)

SEQ ID NO: 1 - protein, 217 aa, Artificial Sequence
APELLGGPSVFLFPPKPKDTLMISRTPEVTCVVVDVSHEDPEVKFNWYVDGVEVHNAKTKPREEQYNSTYRVVSVLTVLHQDWLNGKEYKCKVSNKALPAPIEKTISKAKGQPREPQVYTXPPSRDELTKNQVSLXCXVKGFYPSDIAVEWESNGQPENNYKTTXPVLDSDGSFFLYSXLTVDKSRWQQGNVFSCSVXHEALHNHYTQKSLSLSPGK

SEQ ID NO: 2 - protein, 217 aa, Artificial Sequence
APELLGGPSVFLFPPKPKDTLMISRTPEVTCVVVDVSHEDPEVKFNWYVDGVEVHNAKTKPREEQYNSTYRVVSVLTVLHQDWLNGKEYKCKVSNKALPAPIEKTISKAKGQPREPQVYTSPPSRDELTKNQVSLRCHVKGFYPSDIAVEWESNGQPENNYKTTKPVLDSDGSFFLYSDLTVDKSRWQQGNVFSCSVYHEALHNHYTQKSLSLSPGK

SEQ ID NO: 3 - protein, 65 aa, Artificial Sequence
ITCPPPMSVEHADIWVKSYSLYSRERYICNSGFKRKAGTSSLTECVLNKATNVAHWTTPSLKCIR

SEQ ID NO: 4 - protein, 114 aa, Artificial Sequence
NWVNVISDLKKIEDLIQSMHIDATLYTESDVHPSCKVTAMKCFLLELQVISLESGDASIHDTVENLIILANDSLSSNGNVTESGCKECEELEEKNIKEFLQSFVHIVQMFINTS